European Patent Specification EP 4 061 960 B1, published May 1, 2024. Title: Novel method for pooled intron tagging for real time drug screening. Applicant: CeMM - Forschungszentrum für Molekulare Medizin GmbH. The sequence listing filed with the application follows.

SEQUENCE LISTING (67 sequences)

SEQ ID NO: 1 - RNA, 24 nt, Artificial Sequence
  Primer CROP-seq sgRNA amplicon fwd
atcttgtggaaaggacgaaacacc

SEQ ID NO: 2 - RNA, 23 nt, Artificial Sequence
  Primer CROP-seq sgRNA amplicon rev
tgtctcaagatctagttacgcca

SEQ ID NO: 3 - DNA, 25 bp, Artificial Sequence
  Primer oRT_CROPseq
gactagccttattttaacttgctat

SEQ ID NO: 4 - DNA, 77 bp, Artificial Sequence
  Primer oPD_CROPseq
  modified_base 1: /mod_base="OTHER" /note="phosphorylation"
gttttagagctagaaatagcaagctcctgttcgacacctacccacctcatcccactcttcaaaaggacgaaacaccg

SEQ ID NO: 5 - DNA, 35 bp, Artificial Sequence
  Primer oSBS_CROPseq
cacctcatcccactcttcaaaaggacgaaacaccg

SEQ ID NO: 6 - DNA, 28 bp, Artificial Sequence
  multiplexed amplicon sequencing barcodes FWD1_1
gagaaatcttgtggaaaggacgaaacac

SEQ ID NO: 7 - DNA, 28 bp, Artificial Sequence
  multiplexed amplicon sequencing barcodes FWD1_2
caagaatcttgtggaaaggacgaaacac

SEQ ID NO: 8 - DNA, 28 bp, Artificial Sequence
  multiplexed amplicon sequencing barcodes FWD1_3
gaacaatcttgtggaaaggacgaaacac

SEQ ID NO: 9 - DNA, 28 bp, Artificial Sequence
  v
ccataatcttgtggaaaggacgaaacac

SEQ ID NO: 10 - DNA, 28 bp, Artificial Sequence
  multiplexed amplicon sequencing barcodes FWD1_5
gttagatcttgtggaaaggacgaaacac

SEQ ID NO: 11 - DNA, 28 bp, Artificial Sequence
  multiplexed amplicon sequencing barcodes FWD1_6
actcgatcttgtggaaaggacgaaacac

SEQ ID NO: 12 - DNA, 28 bp, Artificial Sequence
  multiplexed amplicon sequencing barcodes FWD1_7
tgttgatcttgtggaaaggacgaaacac

SEQ ID NO: 13 - DNA, 28 bp, Artificial Sequence
  multiplexed amplicon sequencing barcodes FWD1_8
aggtcatcttgtggaaaggacgaaacac

SEQ ID NO: 14 - DNA, 28 bp, Artificial Sequence
  multiplexed amplicon sequencing barcodes FWD1_9
aggaaatcttgtggaaaggacgaaacac

SEQ ID NO: 15 - DNA, 28 bp, Artificial Sequence
  multiplexed amplicon sequencing barcodes FWD1_10
acagaatcttgtggaaaggacgaaacac

SEQ ID NO: 16 - DNA, 28 bp, Artificial Sequence
  multiplexed amplicon sequencing barcodes FWD1_11
agacaatcttgtggaaaggacgaaacac

SEQ ID NO: 17 - DNA, 28 bp, Artificial Sequence
  multiplexed amplicon sequencing barcodes FWD1_12
tggtaatcttgtggaaaggacgaaacac

SEQ ID NO: 18 - DNA, 28 bp, Artificial Sequence
  multiplexed amplicon sequencing barcodes FWD2_1
ctaggatcttgtggaaaggacgaaacac

SEQ ID NO: 19 - DNA, 28 bp, Artificial Sequence
  multiplexed amplicon sequencing barcodes FWD2_2
cgatgatcttgtggaaaggacgaaacac

SEQ ID NO: 20 - DNA, 28 bp, Artificial Sequence
  multiplexed amplicon sequencing barcodes FWD2_3
ttcgcatcttgtggaaaggacgaaacac

SEQ ID NO: 21 - DNA, 28 bp, Artificial Sequence
  multiplexed amplicon sequencing barcodes FWD2_4
ggttcatcttgtggaaaggacgaaacac

SEQ ID NO: 22 - DNA, 28 bp, Artificial Sequence
  multiplexed amplicon sequencing barcodes FWD2_5
ccgaaatcttgtggaaaggacgaaacac

SEQ ID NO: 23 - DNA, 28 bp, Artificial Sequence
  multiplexed amplicon sequencing barcodes FWD2_6
tcggaatcttgtggaaaggacgaaacac

SEQ ID NO: 24 - DNA, 28 bp, Artificial Sequence
  multiplexed amplicon sequencing barcodes FWD2_7
aagcaatcttgtggaaaggacgaaacac

SEQ ID NO: 25 - DNA, 28 bp, Artificial Sequence
  multiplexed amplicon sequencing barcodes FWD2_8
tcctaatcttgtggaaaggacgaaacac

SEQ ID NO: 26 - DNA, 28 bp, Artificial Sequence
  multiplexed amplicon sequencing barcodes FWD2_9
aatggatcttgtggaaaggacgaaacac

SEQ ID NO: 27 - DNA, 28 bp, Artificial Sequence
  multiplexed amplicon sequencing barcodes FWD2_10
gcatgatcttgtggaaaggacgaaacac

SEQ ID NO: 28 - DNA, 28 bp, Artificial Sequence
  multiplexed amplicon sequencing barcodes FWD2_11
tatgcatcttgtggaaaggacgaaacac

SEQ ID NO: 29 - DNA, 28 bp, Artificial Sequence
  multiplexed amplicon sequencing barcodes FWD2_12
cctgtatcttgtggaaaggacgaaacac

SEQ ID NO: 30 - DNA, 28 bp, Artificial Sequence
  multiplexed amplicon sequencing barcodes FWD3_1
gtggaatcttgtggaaaggacgaaacac

SEQ ID NO: 31 - DNA, 28 bp, Artificial Sequence
  multiplexed amplicon sequencing barcodes FWD3_2
ctgcaatcttgtggaaaggacgaaacac

SEQ ID NO: 32 - DNA, 28 bp, Artificial Sequence
  multiplexed amplicon sequencing barcodes FWD3_3
accaaatcttgtggaaaggacgaaacac

SEQ ID NO: 33 - DNA, 28 bp, Artificial Sequence
  multiplexed amplicon sequencing barcodes FWD3_4
tgcgaatcttgtggaaaggacgaaacac

SEQ ID NO: 34 - DNA, 28 bp, Artificial Sequence
  multiplexed amplicon sequencing barcodes FWD3_5
tgtcaatcttgtggaaaggacgaaacac

SEQ ID NO: 35 - DNA, 28 bp, Artificial Sequence
  multiplexed amplicon sequencing barcodes FWD3_6
tagagatcttgtggaaaggacgaaacac

SEQ ID NO: 36 - DNA, 28 bp, Artificial Sequence
  multiplexed amplicon sequencing barcodes FWD3_7
taccgatcttgtggaaaggacgaaacac

SEQ ID NO: 37 - DNA, 28 bp, Artificial Sequence
  multiplexed amplicon sequencing barcodes FWD3_8
ttgtgatcttgtggaaaggacgaaacac

SEQ ID NO: 38 - DNA, 28 bp, Artificial Sequence
  multiplexed amplicon sequencing barcodes FWD3_9
acaccatcttgtggaaaggacgaaacac

SEQ ID NO: 39 - DNA, 28 bp, Artificial Sequence
  multiplexed amplicon sequencing barcodes FWD3_10
accttatcttgtggaaaggacgaaacac

SEQ ID NO: 40 - DNA, 28 bp, Artificial Sequence
  multiplexed amplicon sequencing barcodes FWD3_11
ctctaatcttgtggaaaggacgaaacac

SEQ ID NO: 41 - DNA, 28 bp, Artificial Sequence
  multiplexed amplicon sequencing barcodes FWD3_12
tcacgatcttgtggaaaggacgaaacac

SEQ ID NO: 42 - DNA, 28 bp, Artificial Sequence
  multiplexed amplicon sequencing barcodes REV1_A
ggcaatgtctcaagatctagttacgcca

SEQ ID NO: 43 - DNA, 28 bp, Artificial Sequence
  multiplexed amplicon sequencing barcodes REV1_B
aacgatgtctcaagatctagttacgcca

SEQ ID NO: 44 - DNA, 28 bp, Artificial Sequence
  multiplexed amplicon sequencing barcodes REV1_C
gtccatgtctcaagatctagttacgcca

SEQ ID NO: 45 - DNA, 28 bp, Artificial Sequence
  multiplexed amplicon sequencing barcodes REV1_D
tgaagtgtctcaagatctagttacgcca

SEQ ID NO: 46 - DNA, 28 bp, Artificial Sequence
  multiplexed amplicon sequencing barcodes REV1_E
gtacgtgtctcaagatctagttacgcca

SEQ ID NO: 47 - DNA, 28 bp, Artificial Sequence
  multiplexed amplicon sequencing barcodes REV1_F
acgtgtgtctcaagatctagttacgcca

SEQ ID NO: 48 - DNA, 28 bp, Artificial Sequence
  multiplexed amplicon sequencing barcodes REV1_G
caacctgtctcaagatctagttacgcca

SEQ ID NO: 49 - DNA, 28 bp, Artificial Sequence
  multiplexed amplicon sequencing barcodes REV1_H
cactttgtctcaagatctagttacgcca

SEQ ID NO: 50 - DNA, 28 bp, Artificial Sequence
  multiplexed amplicon sequencing barcodes REV2_A
cgtaatgtctcaagatctagttacgcca

SEQ ID NO: 51 - DNA, 28 bp, Artificial Sequence
  multiplexed amplicon sequencing barcodes REV2_B
ggtgatgtctcaagatctagttacgcca

SEQ ID NO: 52 - DNA, 28 bp, Artificial Sequence
  multiplexed amplicon sequencing barcodes REV2_C
cctcatgtctcaagatctagttacgcca

SEQ ID NO: 53 - DNA, 28 bp, Artificial Sequence
  multiplexed amplicon sequencing barcodes REV2_D
atgagtgtctcaagatctagttacgcca

SEQ ID NO: 54 - DNA, 28 bp, Artificial Sequence
  multiplexed amplicon sequencing barcodes REV2_E
atccgtgtctcaagatctagttacgcca

SEQ ID NO: 55 - DNA, 28 bp, Artificial Sequence
  multiplexed amplicon sequencing barcodes REV2_F
gactgtgtctcaagatctagttacgcca

SEQ ID NO: 56 - DNA, 28 bp, Artificial Sequence
  multiplexed amplicon sequencing barcodes REV2_G
tctcctgtctcaagatctagttacgcca

SEQ ID NO: 57 - DNA, 28 bp, Artificial Sequence
  multiplexed amplicon sequencing barcodes REV2_H
gctaatgtctcaagatctagttacgcca

SEQ ID NO: 58 - DNA, 28 bp, Artificial Sequence
  multiplexed amplicon sequencing barcodes REV3_A
cttgatgtctcaagatctagttacgcca

SEQ ID NO: 59 - DNA, 28 bp, Artificial Sequence
  multiplexed amplicon sequencing barcodes REV3_B
ggatatgtctcaagatctagttacgcca

SEQ ID NO: 60 - DNA, 28 bp, Artificial Sequence
  multiplexed amplicon sequencing barcodes REV3_C
agtagtgtctcaagatctagttacgcca

SEQ ID NO: 61 - DNA, 28 bp, Artificial Sequence
  multiplexed amplicon sequencing barcodes REV3_D
gatcgtgtctcaagatctagttacgcca

SEQ ID NO: 62 - DNA, 28 bp, Artificial Sequence
  multiplexed amplicon sequencing barcodes REV3_E
agctgtgtctcaagatctagttacgcca

SEQ ID NO: 63 - DNA, 28 bp, Artificial Sequence
  multiplexed amplicon sequencing barcodes REV3_F
cttcctgtctcaagatctagttacgcca

SEQ ID NO: 64 - DNA, 28 bp, Artificial Sequence
  multiplexed amplicon sequencing barcodes REV3_G
attgctgtctcaagatctagttacgcca

SEQ ID NO: 65 - DNA, 28 bp, Artificial Sequence
  multiplexed amplicon sequencing barcodes REV3_H
gtgcttgtctcaagatctagttacgcca

SEQ ID NO: 66 - DNA, 1116 bp, Artificial Sequence
  GFP generic donor plasmid (relevant part)
atgttctttcctgcgttatcccctggagatcgagtgccgcatcaccggctattggtcttactgacatccactttgcctttctctccacagggtggcggtggctcgggcggtggtgggtccggtggcggcggatctggcggtggtggatccgtgagcaagggcgaggagctgttcaccggggtggtgcccatcctggtcgagctggacggcgacgtaaacggccacaagttcagcgtgtccggcgagggcgagggcgatgccacctacggcaagctgaccctgaagttcatctgcaccaccggcaagctgcccgtgccctggcccaccctcgtgaccaccctgacctacggcgtgcagtgcttcagccgctaccccgaccacatgaagcagcacgacttcttcaagtccgccatgcccgaaggctacgtccaggagcgcaccatcttcttcaaggacgacggcaactacaagacccgcgccgaggtgaagttcgagggcgacaccctggtgaaccgcatcgagctgaagggcatcgacttcaaggaggacggcaacatcctggggcacaagctggagtacaactacaacagccacaacgtctatatcatggccgacaagcagaagaacggcatcaaggtgaacttcaagatccgccacaacatcgaggacggcagcgtgcagctcgccgaccactaccagcagaacacccccatcggcgacggccccgtgctgctgcccgacaaccactacctgagcacccagtccgccctgagcaaagaccccaacgagaagcgcgatcacatggtcctgctggagttcgtgaccgccgccgggatcactctcggcatggacgagctgtacaagggcggcggtggatccggtggcggcggatctggcggtggaggttcgggtggcggtgggtcgggcaaggtaagtatcaattagaagacgaattcccggtgatgcggcactcgatctcgaattcttacagacaagctgtgaccgtctccgggagctgcatgtgtcagaggttttcaccgtcatcaccgaaacgcgcgagacgaaagggcctcgtgatacgcctatttttataggttaatgtcatgataataatgg

SEQ ID NO: 67 - DNA, 5071 bp, Artificial Sequence
  GFP minicircle
acattaccctgttatccctagatacattaccctgttatcccagatgacataccctgttatccctagatgacattaccctgttatcccagatgacattaccctgttatccctagatacattaccctgttatcccagatgacataccctgttatccctagatgacattaccctgttatcccagatgacattaccctgttatccctagatacattaccctgttatcccagatgacataccctgttatccctagatgacattaccctgttatcccagatgacattaccctgttatccctagatacattaccctgttatcccagatgacataccctgttatccctagatgacattaccctgttatcccagatgacattaccctgttatccctagatacattaccctgttatcccagatgacataccctgttatccctagatgacattaccctgttatcccagatgacattaccctgttatccctagatacattaccctgttatcccagatgacataccctgttatccctagatgacattaccctgttatcccagatgacattaccctgttatccctagatacattaccctgttatcccagatgacataccctgttatccctagatgacattaccctgttatcccagatgacattaccctgttatccctagatacattaccctgttatcccagatgacataccctgttatccctagatgacattaccctgttatcccagataaactcaatgatgatgatgatgatggtcgagactcagcggccgcggtgccagggcgtgcccttgggctccccgggcgcgactagtgaattcagatctgatcctgcgttatcccctggagatcgagtgccgcatcaccggctattggtcttactgacatccactttgcctttctctccacagggtggcggtggctcgggcggtggtgggtccggtggcggcggatctggcggtggtggatccgtgagcaagggcgaggagctgttcaccggggtggtgcccatcctggtcgagctggacggcgacgtaaacggccacaagttcagcgtgtccggcgagggcgagggcgatgccacctacggcaagctgaccctgaagttcatctgcaccaccggcaagctgcccgtgccctggcccaccctcgtgaccaccctgacctacggcgtgcagtgcttcagccgctaccccgaccacatgaagcagcacgacttcttcaagtccgccatgcccgaaggctacgtccaggagcgcaccatcttcttcaaggacgacggcaactacaagacccgcgccgaggtgaagttcgagggcgacaccctggtgaaccgcatcgagctgaagggcatcgacttcaaggaggacggcaacatcctggggcacaagctggagtacaactacaacagccacaacgtctatatcatggccgacaagcagaagaacggcatcaaggtgaacttcaagatccgccacaacatcgaggacggcagcgtgcagctcgccgaccactaccagcagaacacccccatcggcgacggccccgtgctgctgcccgacaaccactacctgagcacccagtccgccctgagcaaagaccccaacgagaagcgcgatcacatggtcctgctggagttcgtgaccgccgccgggatcactctcggcatggacgagctgtacaagggcggcggtggatccggtggcggcggatctggcggtggaggttcgggtggcggtgggtcgggcaaggtaagtatcaattagaagacgaattccatctctagagtcgacccatgggggcccgccccaactggggtaacctttgagttctctcagttgggggtaatcagcatcatgatgtggtaccacatcatgatgctgattataagaatgcggccgccacactctagtggatctcgagttaataattcagaagaactcgtcaagaaggcgatagaaggcgatgcgctgcgaatcgggagcggcgataccgtaaagcacgaggaagcggtcagcccattcgccgccaagctcttcagcaatatcacgggtagccaacgctatgtcctgatagcggtccgccacacccagccggccacagtcgatgaatccagaaaagcggccattttccaccatgatattcggcaagcaggcatcgccatgggtcacgacgagatcctcgccgtcgggcatgctcgccttgagcctggcgaacagttcggctggcgcgagcccctgatgctcttcgtccagatcatcctgatcgacaagaccggcttccatccgagtacgtgctcgctcgatgcgatgtttcgcttggtggtcgaatgggcaggtagccggatcaagcgtatgcagccgccgcattgcatcagccatgatggatactttctcggcaggagcaaggtgagatgacaggagatcctgccccggcacttcgcccaatagcagccagtcccttcccgcttcagtgacaacgtcgagcacagctgcgcaaggaacgcccgtcgtggccagccacgatagccgcgctgcctcgtcttgcagttcattcagggcaccggacaggtcggtcttgacaaaaagaaccgggcgcccctgcgctgacagccggaacacggcggcatcagagcagccgattgtctgttgtgcccagtcatagccgaatagcctctccacccaagcggccggagaacctgcgtgcaatccatcttgttcaatcatgcgaaacgatcctcatcctgtctcttgatcagagcttgatcccctgcgccatcagatccttggcggcgagaaagccatccagtttactttgcagggcttcccaaccttaccagagggcgccccagctggcaattccggttcgcttgctgtccataaaaccgcccagtctagctatcgccatgtaagcccactgcaagctacctgctttctctttgcgcttgcgttttcccttgtccagatagcccagtagctgacattcatccggggtcagcaccgtttctgcggactggctttctacgtgctcgaggggggccaaacggtctccagcttggctgttttggcggatgagagaagattttcagcctgatacagattaaatcagaacgcagaagcggtctgataaaacagaatttgcctggcggcagtagcgcggtggtcccacctgaccccatgccgaactcagaagtgaaacgccgtagcgccgatggtagtgtggggtctccccatgcgagagtagggaactgccaggcatcaaataaaacgaaaggctcagtcgaaagactgggcctttcgttttatctgttgtttgtcggtgaacgctctcctgagtaggacaaatccgccgggagcggatttgaacgttgcgaagcaacggcccggagggtggcgggcaggacgcccgccataaactgccaggcatcaaattaagcagaaggccatcctgacggatggcctttttgcgtttctacaaactcttttgtttatttttctaaatacattcaaatatgtatccgctcatgaccaaaatcccttaacgtgagttttcgttccactgagcgtcagaccccgtagaaaagatcaaaggatcttcttgagatcctttttttctgcgcgtaatctgctgcttgcaaacaaaaaaaccaccgctaccagcggtggtttgtttgccggatcaagagctaccaactctttttccgaaggtaactggcttcagcagagcgcagataccaaatactgtccttctagtgtagccgtagttaggccaccacttcaagaactctgtagcaccgcctacatacctcgctctgctaatcctgttaccagtggctgctgccagtggcgataagtcgtgtcttaccgggttggactcaagacgatagttaccggataaggcgcagcggtcgggctgaacggggggttcgtgcacacagcccagcttggagcgaacgacctacaccgaactgagatacctacagcgtgagctatgagaaagcgccacgcttcccgaagggagaaaggcggacaggtatccggtaagcggcagggtcggaacaggagagcgcacgagggagcttccagggggaaacgcctggtatctttatagtcctgtcgggtttcgccacctctgacttgagcgtcgatttttgtgatgctcgtcaggggggcggagcctatggaaaaacgccagcaacgcggcctttttacggttcctggccttttgctggccttttgctcacatgttctttcctgcgttatcccctgattctgtggataaccgtattaccgcctttgagtgagctgataccgctcgccgcagccgaacgaccgagcgcagcgagtcagtgagcgaggaagcggaagagcgcctgatgcggtattttctccttacgcatctgtgcggtatttcacaccgcatatggtgcactctcagtacaatctgctctgatgccgcatagttaagccagtatacactccgctatcgctacgtgactgggtcatggctgcgccccgacacccgccaacacccgctgacgcgccctgacgggcttgtctgctcccggcatccgcttacagacaagctgtgaccgtctccgggagctgcatgtgtcagaggttttcaccgtcatcaccgaaacgcgcgaggcagcagatcaattcgcgcgcgaaggcgaagcggcatgcataatgtgcctgtcaaatggacgaagcagggattctgcaaaccctatgctactccgtcaagccgtcaattgtctgattcgttaccaattatgacaacttgacggctacatcattcactttttcttcacaaccggcacggaactcgctcgggctggccccggtgcattttttaaatacccgcgagaaatagagttgatcgtcaaaaccaacattgcgaccgacggtggcgataggcatccgggtggtgctcaaaagcagcttcgcctggctgatacgttggtcctcgcgccagcttaagacgctaatccctaactgctggcggaaaagatgtgacagacgcgacggcgacaagcaaacatgctgtgcgacgctggcgat